European Patent Specification EP 3 688 175 B1, published March 13, 2024. Title: Genetically Modified Isopropylmalate Isomerase Enzyme Complexes and Processes to Prepare Elongated 2-Ketoacids and C5-C10 Compounds Therewith. Applicant: The Dow Chemical Company Sanghani, Paresh Shiue, Eric C. Greenwalt, Scott A. The sequence listing filed with the application follows.

SEQUENCE LISTING (40 sequences)

SEQ ID NO: 1 - protein, 466 aa, Escherichia coli
MAKTLYEKLFDAHVVYEAENETPLLYIDRHLVHEVTSPQAFDGLRAHGRPVRQPGKTFATMDHNVSTQTKDINACGEMARIQMQELIKNCKEFGVELYDLNHPYQGIVHVMGPEQGVTLPGMTIVCGDSHTATHGAFGALAFGIGTSEVEHVLATQTLKQGRAKTMKIEVQGKAAPGITAKDIVLAIIGKTGSAGGTGHVVEFCGEAIRDLSMEGRMTLCNMAIEMGAKAGLVAPDETTFNYVKGRLHAPKGKDFDDAVAYWKTLQTDEGATFDTVVTLQAEEISPQVTWGTNPGQVISVNDNIPDPASFADPVERASAEKALAYMGLKPGIPLTEVAIDKVFIGSCTNSRIEDLRAAAEIAKGRKVAPGVQALVVPGSGPVKAQAEAEGLDKIFIEAGFEWRLPGCSMCLAMNNDRLNPGERCASTSNRNFEGRQGRGGRTHLVSPAMAAAAAVTGHFADIRNIK

SEQ ID NO: 2 - protein, 201 aa, Escherichia coli
MAEKFIKHTGLVVPLDAANVDTDAIIPKQFLQKVTRTGFGAHLFNDWRFLDEKGQQPNPDFVLNFPQYQGASILLARENFGCGSSREHAPWALTDYGFKVVIAPSFADIFYGNSFNNQLLPVKLSDAEVDELFALVKANPGIHFDVDLEAQEVKAGEKTYRFTIDAFRRHCMMNGLDSIGLTLQHDDAIAAYEAKQPAFMN

SEQ ID NO: 3 - protein, 466 aa, Artificial Sequence
  Synthesized - Modified LeuC (V35A)
MAKTLYEKLFDAHVVYEAENETPLLYIDRHLVHEATSPQAFDGLRAHGRPVRQPGKTFATMDHNVSTQTKDINACGEMARIQMQELIKNCKEFGVELYDLNHPYQGIVHVMGPEQGVTLPGMTIVCGDSHTATHGAFGALAFGIGTSEVEHVLATQTLKQGRAKTMKIEVQGKAAPGITAKDIVLAIIGKTGSAGGTGHVVEFCGEAIRDLSMEGRMTLCNMAIEMGAKAGLVAPDETTFNYVKGRLHAPKGKDFDDAVAYWKTLQTDEGATFDTVVTLQAEEISPQVTWGTNPGQVISVNDNIPDPASFADPVERASAEKALAYMGLKPGIPLTEVAIDKVFIGSCTNSRIEDLRAAAEIAKGRKVAPGVQALVVPGSGPVKAQAEAEGLDKIFIEAGFEWRLPGCSMCLAMNNDRLNPGERCASTSNRNFEGRQGRGGRTHLVSPAMAAAAAVTGHFADIRNIK

SEQ ID NO: 4 - protein, 466 aa, Artificial Sequence
  Synthesized - Modified LeuC (V35G)
MAKTLYEKLFDAHVVYEAENETPLLYIDRHLVHEGTSPQAFDGLRAHGRPVRQPGKTFATMDHNVSTQTKDINACGEMARIQMQELIKNCKEFGVELYDLNHPYQGIVHVMGPEQGVTLPGMTIVCGDSHTATHGAFGALAFGIGTSEVEHVLATQTLKQGRAKTMKIEVQGKAAPGITAKDIVLAIIGKTGSAGGTGHVVEFCGEAIRDLSMEGRMTLCNMAIEMGAKAGLVAPDETTFNYVKGRLHAPKGKDFDDAVAYWKTLQTDEGATFDTVVTLQAEEISPQVTWGTNPGQVISVNDNIPDPASFADPVERASAEKALAYMGLKPGIPLTEVAIDKVFIGSCTNSRIEDLRAAAEIAKGRKVAPGVQALVVPGSGPVKAQAEAEGLDKIFIEAGFEWRLPGCSMCLAMNNDRLNPGERCASTSNRNFEGRQGRGGRTHLVSPAMAAAAAVTGHFADIRNIK

SEQ ID NO: 5 - protein, 466 aa, Artificial Sequence
  Synthezied - Modified LeuC (L411A)
MAKTLYEKLFDAHVVYEAENETPLLYIDRHLVHEVTSPQAFDGLRAHGRPVRQPGKTFATMDHNVSTQTKDINACGEMARIQMQELIKNCKEFGVELYDLNHPYQGIVHVMGPEQGVTLPGMTIVCGDSHTATHGAFGALAFGIGTSEVEHVLATQTLKQGRAKTMKIEVQGKAAPGITAKDIVLAIIGKTGSAGGTGHVVEFCGEAIRDLSMEGRMTLCNMAIEMGAKAGLVAPDETTFNYVKGRLHAPKGKDFDDAVAYWKTLQTDEGATFDTVVTLQAEEISPQVTWGTNPGQVISVNDNIPDPASFADPVERASAEKALAYMGLKPGIPLTEVAIDKVFIGSCTNSRIEDLRAAAEIAKGRKVAPGVQALVVPGSGPVKAQAEAEGLDKIFIEAGFEWRLPGCSMCAAMNNDRLNPGERCASTSNRNFEGRQGRGGRTHLVSPAMAAAAAVTGHFADIRNIK

SEQ ID NO: 6 - protein, 466 aa, Artificial Sequence
  Synthesized - Modified LeuC (L411G)
MAKTLYEKLFDAHVVYEAENETPLLYIDRHLVHEVTSPQAFDGLRAHGRPVRQPGKTFATMDHNVSTQTKDINACGEMARIQMQELIKNCKEFGVELYDLNHPYQGIVHVMGPEQGVTLPGMTIVCGDSHTATHGAFGALAFGIGTSEVEHVLATQTLKQGRAKTMKIEVQGKAAPGITAKDIVLAIIGKTGSAGGTGHVVEFCGEAIRDLSMEGRMTLCNMAIEMGAKAGLVAPDETTFNYVKGRLHAPKGKDFDDAVAYWKTLQTDEGATFDTVVTLQAEEISPQVTWGTNPGQVISVNDNIPDPASFADPVERASAEKALAYMGLKPGIPLTEVAIDKVFIGSCTNSRIEDLRAAAEIAKGRKVAPGVQALVVPGSGPVKAQAEAEGLDKIFIEAGFEWRLPGCSMCGAMNNDRLNPGERCASTSNRNFEGRQGRGGRTHLVSPAMAAAAAVTGHFADIRNIK

SEQ ID NO: 7 - protein, 466 aa, Artificial Sequence
  Synthesized - Modified LeuC (L411V)
MAKTLYEKLFDAHVVYEAENETPLLYIDRHLVHEVTSPQAFDGLRAHGRPVRQPGKTFATMDHNVSTQTKDINACGEMARIQMQELIKNCKEFGVELYDLNHPYQGIVHVMGPEQGVTLPGMTIVCGDSHTATHGAFGALAFGIGTSEVEHVLATQTLKQGRAKTMKIEVQGKAAPGITAKDIVLAIIGKTGSAGGTGHVVEFCGEAIRDLSMEGRMTLCNMAIEMGAKAGLVAPDETTFNYVKGRLHAPKGKDFDDAVAYWKTLQTDEGATFDTVVTLQAEEISPQVTWGTNPGQVISVNDNIPDPASFADPVERASAEKALAYMGLKPGIPLTEVAIDKVFIGSCTNSRIEDLRAAAEIAKGRKVAPGVQALVVPGSGPVKAQAEAEGLDKIFIEAGFEWRLPGCSMCVAMNNDRLNPGERCASTSNRNFEGRQGRGGRTHLVSPAMAAAAAVTGHFADIRNIK

SEQ ID NO: 8 - protein, 466 aa, Artificial Sequence
  Synthesized - Modified LeuC (V35A L411A)
MAKTLYEKLFDAHVVYEAENETPLLYIDRHLVHEATSPQAFDGLRAHGRPVRQPGKTFATMDHNVSTQTKDINACGEMARIQMQELIKNCKEFGVELYDLNHPYQGIVHVMGPEQGVTLPGMTIVCGDSHTATHGAFGALAFGIGTSEVEHVLATQTLKQGRAKTMKIEVQGKAAPGITAKDIVLAIIGKTGSAGGTGHVVEFCGEAIRDLSMEGRMTLCNMAIEMGAKAGLVAPDETTFNYVKGRLHAPKGKDFDDAVAYWKTLQTDEGATFDTVVTLQAEEISPQVTWGTNPGQVISVNDNIPDPASFADPVERASAEKALAYMGLKPGIPLTEVAIDKVFIGSCTNSRIEDLRAAAEIAKGRKVAPGVQALVVPGSGPVKAQAEAEGLDKIFIEAGFEWRLPGCSMCAAMNNDRLNPGERCASTSNRNFEGRQGRGGRTHLVSPAMAAAAAVTGHFADIRNIK

SEQ ID NO: 9 - protein, 466 aa, Artificial Sequence
  Synthesized - Modified LeuC (V35A L411G)
MAKTLYEKLFDAHVVYEAENETPLLYIDRHLVHEATSPQAFDGLRAHGRPVRQPGKTFATMDHNVSTQTKDINACGEMARIQMQELIKNCKEFGVELYDLNHPYQGIVHVMGPEQGVTLPGMTIVCGDSHTATHGAFGALAFGIGTSEVEHVLATQTLKQGRAKTMKIEVQGKAAPGITAKDIVLAIIGKTGSAGGTGHVVEFCGEAIRDLSMEGRMTLCNMAIEMGAKAGLVAPDETTFNYVKGRLHAPKGKDFDDAVAYWKTLQTDEGATFDTVVTLQAEEISPQVTWGTNPGQVISVNDNIPDPASFADPVERASAEKALAYMGLKPGIPLTEVAIDKVFIGSCTNSRIEDLRAAAEIAKGRKVAPGVQALVVPGSGPVKAQAEAEGLDKIFIEAGFEWRLPGCSMCGAMNNDRLNPGERCASTSNRNFEGRQGRGGRTHLVSPAMAAAAAVTGHFADIRNIK

SEQ ID NO: 10 - protein, 466 aa, Artificial Sequence
  Synthesized - Modified LeuC (V35A L411V)
MAKTLYEKLFDAHVVYEAENETPLLYIDRHLVHEATSPQAFDGLRAHGRPVRQPGKTFATMDHNVSTQTKDINACGEMARIQMQELIKNCKEFGVELYDLNHPYQGIVHVMGPEQGVTLPGMTIVCGDSHTATHGAFGALAFGIGTSEVEHVLATQTLKQGRAKTMKIEVQGKAAPGITAKDIVLAIIGKTGSAGGTGHVVEFCGEAIRDLSMEGRMTLCNMAIEMGAKAGLVAPDETTFNYVKGRLHAPKGKDFDDAVAYWKTLQTDEGATFDTVVTLQAEEISPQVTWGTNPGQVISVNDNIPDPASFADPVERASAEKALAYMGLKPGIPLTEVAIDKVFIGSCTNSRIEDLRAAAEIAKGRKVAPGVQALVVPGSGPVKAQAEAEGLDKIFIEAGFEWRLPGCSMCVAMNNDRLNPGERCASTSNRNFEGRQGRGGRTHLVSPAMAAAAAVTGHFADIRNIK

SEQ ID NO: 11 - protein, 466 aa, Artificial Sequence
  Synthesized - Modified LeuC (V35G L411A)
MAKTLYEKLFDAHVVYEAENETPLLYIDRHLVHEGTSPQAFDGLRAHGRPVRQPGKTFATMDHNVSTQTKDINACGEMARIQMQELIKNCKEFGVELYDLNHPYQGIVHVMGPEQGVTLPGMTIVCGDSHTATHGAFGALAFGIGTSEVEHVLATQTLKQGRAKTMKIEVQGKAAPGITAKDIVLAIIGKTGSAGGTGHVVEFCGEAIRDLSMEGRMTLCNMAIEMGAKAGLVAPDETTFNYVKGRLHAPKGKDFDDAVAYWKTLQTDEGATFDTVVTLQAEEISPQVTWGTNPGQVISVNDNIPDPASFADPVERASAEKALAYMGLKPGIPLTEVAIDKVFIGSCTNSRIEDLRAAAEIAKGRKVAPGVQALVVPGSGPVKAQAEAEGLDKIFIEAGFEWRLPGCSMCAAMNNDRLNPGERCASTSNRNFEGRQGRGGRTHLVSPAMAAAAAVTGHFADIRNIK

SEQ ID NO: 12 - protein, 466 aa, Artificial Sequence
  Synthesized - Modified LeuC (V35G L411G)
MAKTLYEKLFDAHVVYEAENETPLLYIDRHLVHEGTSPQAFDGLRAHGRPVRQPGKTFATMDHNVSTQTKDINACGEMARIQMQELIKNCKEFGVELYDLNHPYQGIVHVMGPEQGVTLPGMTIVCGDSHTATHGAFGALAFGIGTSEVEHVLATQTLKQGRAKTMKIEVQGKAAPGITAKDIVLAIIGKTGSAGGTGHVVEFCGEAIRDLSMEGRMTLCNMAIEMGAKAGLVAPDETTFNYVKGRLHAPKGKDFDDAVAYWKTLQTDEGATFDTVVTLQAEEISPQVTWGTNPGQVISVNDNIPDPASFADPVERASAEKALAYMGLKPGIPLTEVAIDKVFIGSCTNSRIEDLRAAAEIAKGRKVAPGVQALVVPGSGPVKAQAEAEGLDKIFIEAGFEWRLPGCSMCGAMNNDRLNPGERCASTSNRNFEGRQGRGGRTHLVSPAMAAAAAVTGHFADIRNIK

SEQ ID NO: 13 - protein, 466 aa, Artificial Sequence
  Synthesized - Modified LeuC (V35G L411V)
MAKTLYEKLFDAHVVYEAENETPLLYIDRHLVHEGTSPQAFDGLRAHGRPVRQPGKTFATMDHNVSTQTKDINACGEMARIQMQELIKNCKEFGVELYDLNHPYQGIVHVMGPEQGVTLPGMTIVCGDSHTATHGAFGALAFGIGTSEVEHVLATQTLKQGRAKTMKIEVQGKAAPGITAKDIVLAIIGKTGSAGGTGHVVEFCGEAIRDLSMEGRMTLCNMAIEMGAKAGLVAPDETTFNYVKGRLHAPKGKDFDDAVAYWKTLQTDEGATFDTVVTLQAEEISPQVTWGTNPGQVISVNDNIPDPASFADPVERASAEKALAYMGLKPGIPLTEVAIDKVFIGSCTNSRIEDLRAAAEIAKGRKVAPGVQALVVPGSGPVKAQAEAEGLDKIFIEAGFEWRLPGCSMCVAMNNDRLNPGERCASTSNRNFEGRQGRGGRTHLVSPAMAAAAAVTGHFADIRNIK

SEQ ID NO: 14 - protein, 201 aa, Artificial Sequence
  Synthesized - Modified LeuD (H88A)
MAEKFIKHTGLVVPLDAANVDTDAIIPKQFLQKVTRTGFGAHLFNDWRFLDEKGQQPNPDFVLNFPQYQGASILLARENFGCGSSREAAPWALTDYGFKVVIAPSFADIFYGNSFNNQLLPVKLSDAEVDELFALVKANPGIHFDVDLEAQEVKAGEKTYRFTIDAFRRHCMMNGLDSIGLTLQHDDAIAAYEAKQPAFMN

SEQ ID NO: 15 - protein, 201 aa, Artificial Sequence
  Synthesized - Modified LeuD (H88G)
MAEKFIKHTGLVVPLDAANVDTDAIIPKQFLQKVTRTGFGAHLFNDWRFLDEKGQQPNPDFVLNFPQYQGASILLARENFGCGSSREGAPWALTDYGFKVVIAPSFADIFYGNSFNNQLLPVKLSDAEVDELFALVKANPGIHFDVDLEAQEVKAGEKTYRFTIDAFRRHCMMNGLDSIGLTLQHDDAIAAYEAKQPAFMN

SEQ ID NO: 16 - protein, 201 aa, Artificial Sequence
  Synthesized - Modified LeuD (H88V)
MAEKFIKHTGLVVPLDAANVDTDAIIPKQFLQKVTRTGFGAHLFNDWRFLDEKGQQPNPDFVLNFPQYQGASILLARENFGCGSSREVAPWALTDYGFKVVIAPSFADIFYGNSFNNQLLPVKLSDAEVDELFALVKANPGIHFDVDLEAQEVKAGEKTYRFTIDAFRRHCMMNGLDSIGLTLQHDDAIAAYEAKQPAFMN

SEQ ID NO: 17 - protein, 201 aa, Artificial Sequence
  Synthesized - Modified LeuD (H88S)
MAEKFIKHTGLVVPLDAANVDTDAIIPKQFLQKVTRTGFGAHLFNDWRFLDEKGQQPNPDFVLNFPQYQGASILLARENFGCGSSRESAPWALTDYGFKVVIAPSFADIFYGNSFNNQLLPVKLSDAEVDELFALVKANPGIHFDVDLEAQEVKAGEKTYRFTIDAFRRHCMMNGLDSIGLTLQHDDAIAAYEAKQPAFMN

SEQ ID NO: 18 - protein, 201 aa, Artificial Sequence
  Synthesized - Modified LeuD (L31A)
MAEKFIKHTGLVVPLDAANVDTDAIIPKQFAQKVTRTGFGAHLFNDWRFLDEKGQQPNPDFVLNFPQYQGASILLARENFGCGSSREHAPWALTDYGFKVVIAPSFADIFYGNSFNNQLLPVKLSDAEVDELFALVKANPGIHFDVDLEAQEVKAGEKTYRFTIDAFRRHCMMNGLDSIGLTLQHDDAIAAYEAKQPAFMN

SEQ ID NO: 19 - protein, 201 aa, Artificial Sequence
  Synthesized - Modified LeuD (L31A H88A)
MAEKFIKHTGLVVPLDAANVDTDAIIPKQFAQKVTRTGFGAHLFNDWRFLDEKGQQPNPDFVLNFPQYQGASILLARENFGCGSSREAAPWALTDYGFKVVIAPSFADIFYGNSFNNQLLPVKLSDAEVDELFALVKANPGIHFDVDLEAQEVKAGEKTYRFTIDAFRRHCMMNGLDSIGLTLQHDDAIAAYEAKQPAFMN

SEQ ID NO: 20 - protein, 201 aa, Artificial Sequence
  Synthesized - Modified LeuD (L31A H88G)
MAEKFIKHTGLVVPLDAANVDTDAIIPKQFAQKVTRTGFGAHLFNDWRFLDEKGQQPNPDFVLNFPQYQGASILLARENFGCGSSREGAPWALTDYGFKVVIAPSFADIFYGNSFNNQLLPVKLSDAEVDELFALVKANPGIHFDVDLEAQEVKAGEKTYRFTIDAFRRHCMMNGLDSIGLTLQHDDAIAAYEAKQPAFMN

SEQ ID NO: 21 - protein, 201 aa, Artificial Sequence
  Synthesized - Modified LeuD (L31A H88V)
MAEKFIKHTGLVVPLDAANVDTDAIIPKQFAQKVTRTGFGAHLFNDWRFLDEKGQQPNPDFVLNFPQYQGASILLARENFGCGSSREVAPWALTDYGFKVVIAPSFADIFYGNSFNNQLLPVKLSDAEVDELFALVKANPGIHFDVDLEAQEVKAGEKTYRFTIDAFRRHCMMNGLDSIGLTLQHDDAIAAYEAKQPAFMN

SEQ ID NO: 22 - protein, 201 aa, Artificial Sequence
  Synthesized - Modified LeuD (L31A H88S)
MAEKFIKHTGLVVPLDAANVDTDAIIPKQFAQKVTRTGFGAHLFNDWRFLDEKGQQPNPDFVLNFPQYQGASILLARENFGCGSSRESAPWALTDYGFKVVIAPSFADIFYGNSFNNQLLPVKLSDAEVDELFALVKANPGIHFDVDLEAQEVKAGEKTYRFTIDAFRRHCMMNGLDSIGLTLQHDDAIAAYEAKQPAFMN

SEQ ID NO: 23 - protein, 201 aa, Artificial Sequence
  Synthesized - Modified LeuD (L31G)
MAEKFIKHTGLVVPLDAANVDTDAIIPKQFGQKVTRTGFGAHLFNDWRFLDEKGQQPNPDFVLNFPQYQGASILLARENFGCGSSREHAPWALTDYGFKVVIAPSFADIFYGNSFNNQLLPVKLSDAEVDELFALVKANPGIHFDVDLEAQEVKAGEKTYRFTIDAFRRHCMMNGLDSIGLTLQHDDAIAAYEAKQPAFMN

SEQ ID NO: 24 - protein, 201 aa, Artificial Sequence
  Synthesized - Modified LeuD (L31G H88A)
MAEKFIKHTGLVVPLDAANVDTDAIIPKQFGQKVTRTGFGAHLFNDWRFLDEKGQQPNPDFVLNFPQYQGASILLARENFGCGSSREAAPWALTDYGFKVVIAPSFADIFYGNSFNNQLLPVKLSDAEVDELFALVKANPGIHFDVDLEAQEVKAGEKTYRFTIDAFRRHCMMNGLDSIGLTLQHDDAIAAYEAKQPAFMN

SEQ ID NO: 25 - protein, 201 aa, Artificial Sequence
  Synthesized - Modified LeuD (L31G H88G)
MAEKFIKHTGLVVPLDAANVDTDAIIPKQFGQKVTRTGFGAHLFNDWRFLDEKGQQPNPDFVLNFPQYQGASILLARENFGCGSSREGAPWALTDYGFKVVIAPSFADIFYGNSFNNQLLPVKLSDAEVDELFALVKANPGIHFDVDLEAQEVKAGEKTYRFTIDAFRRHCMMNGLDSIGLTLQHDDAIAAYEAKQPAFMN

SEQ ID NO: 26 - protein, 201 aa, Artificial Sequence
  Synthesized - Modified LeuD (L31G H88V)
MAEKFIKHTGLVVPLDAANVDTDAIIPKQFGQKVTRTGFGAHLFNDWRFLDEKGQQPNPDFVLNFPQYQGASILLARENFGCGSSREVAPWALTDYGFKVVIAPSFADIFYGNSFNNQLLPVKLSDAEVDELFALVKANPGIHFDVDLEAQEVKAGEKTYRFTIDAFRRHCMMNGLDSIGLTLQHDDAIAAYEAKQPAFMN

SEQ ID NO: 27 - protein, 201 aa, Artificial Sequence
  Synthesized - Modified LeuD( L31G H88S)
MAEKFIKHTGLVVPLDAANVDTDAIIPKQFGQKVTRTGFGAHLFNDWRFLDEKGQQPNPDFVLNFPQYQGASILLARENFGCGSSRESAPWALTDYGFKVVIAPSFADIFYGNSFNNQLLPVKLSDAEVDELFALVKANPGIHFDVDLEAQEVKAGEKTYRFTIDAFRRHCMMNGLDSIGLTLQHDDAIAAYEAKQPAFMN

SEQ ID NO: 28 - protein, 201 aa, Artificial Sequence
  Synthesized - Modified LeuD (L31V)
MAEKFIKHTGLVVPLDAANVDTDAIIPKQFVQKVTRTGFGAHLFNDWRFLDEKGQQPNPDFVLNFPQYQGASILLARENFGCGSSREHAPWALTDYGFKVVIAPSFADIFYGNSFNNQLLPVKLSDAEVDELFALVKANPGIHFDVDLEAQEVKAGEKTYRFTIDAFRRHCMMNGLDSIGLTLQHDDAIAAYEAKQPAFMN

SEQ ID NO: 29 - protein, 201 aa, Artificial Sequence
  Synthesized - Modified LeuD (L31V H88A)
MAEKFIKHTGLVVPLDAANVDTDAIIPKQFVQKVTRTGFGAHLFNDWRFLDEKGQQPNPDFVLNFPQYQGASILLARENFGCGSSREAAPWALTDYGFKVVIAPSFADIFYGNSFNNQLLPVKLSDAEVDELFALVKANPGIHFDVDLEAQEVKAGEKTYRFTIDAFRRHCMMNGLDSIGLTLQHDDAIAAYEAKQPAFMN

SEQ ID NO: 30 - protein, 201 aa, Artificial Sequence
  Synthesized - Modified LeuD (L31V H88G)
MAEKFIKHTGLVVPLDAANVDTDAIIPKQFVQKVTRTGFGAHLFNDWRFLDEKGQQPNPDFVLNFPQYQGASILLARENFGCGSSREGAPWALTDYGFKVVIAPSFADIFYGNSFNNQLLPVKLSDAEVDELFALVKANPGIHFDVDLEAQEVKAGEKTYRFTIDAFRRHCMMNGLDSIGLTLQHDDAIAAYEAKQPAFMN

SEQ ID NO: 31 - protein, 201 aa, Artificial Sequence
  Synthesized - Modified LeuD (L31V H88V)
MAEKFIKHTGLVVPLDAANVDTDAIIPKQFVQKVTRTGFGAHLFNDWRFLDEKGQQPNPDFVLNFPQYQGASILLARENFGCGSSREVAPWALTDYGFKVVIAPSFADIFYGNSFNNQLLPVKLSDAEVDELFALVKANPGIHFDVDLEAQEVKAGEKTYRFTIDAFRRHCMMNGLDSIGLTLQHDDAIAAYEAKQPAFMN

SEQ ID NO: 32 - protein, 201 aa, Artificial Sequence
  Synthesized - Modified LeuD (L31V H88S)
MAEKFIKHTGLVVPLDAANVDTDAIIPKQFVQKVTRTGFGAHLFNDWRFLDEKGQQPNPDFVLNFPQYQGASILLARENFGCGSSRESAPWALTDYGFKVVIAPSFADIFYGNSFNNQLLPVKLSDAEVDELFALVKANPGIHFDVDLEAQEVKAGEKTYRFTIDAFRRHCMMNGLDSIGLTLQHDDAIAAYEAKQPAFMN

SEQ ID NO: 33 - protein, 201 aa, Artificial Sequence
  Synthesized - Modified LeuD (L31S)
MAEKFIKHTGLVVPLDAANVDTDAIIPKQFSQKVTRTGFGAHLFNDWRFLDEKGQQPNPDFVLNFPQYQGASILLARENFGCGSSREHAPWALTDYGFKVVIAPSFADIFYGNSFNNQLLPVKLSDAEVDELFALVKANPGIHFDVDLEAQEVKAGEKTYRFTIDAFRRHCMMNGLDSIGLTLQHDDAIAAYEAKQPAFMN

SEQ ID NO: 34 - protein, 201 aa, Artificial Sequence
  Synthesized - Modified LeuD (L31S H88A)
MAEKFIKHTGLVVPLDAANVDTDAIIPKQFSQKVTRTGFGAHLFNDWRFLDEKGQQPNPDFVLNFPQYQGASILLARENFGCGSSREAAPWALTDYGFKVVIAPSFADIFYGNSFNNQLLPVKLSDAEVDELFALVKANPGIHFDVDLEAQEVKAGEKTYRFTIDAFRRHCMMNGLDSIGLTLQHDDAIAAYEAKQPAFMN

SEQ ID NO: 35 - protein, 201 aa, Artificial Sequence
  Synthesized - Modified LeuD (L31S H88G)
MAEKFIKHTGLVVPLDAANVDTDAIIPKQFSQKVTRTGFGAHLFNDWRFLDEKGQQPNPDFVLNFPQYQGASILLARENFGCGSSREGAPWALTDYGFKVVIAPSFADIFYGNSFNNQLLPVKLSDAEVDELFALVKANPGIHFDVDLEAQEVKAGEKTYRFTIDAFRRHCMMNGLDSIGLTLQHDDAIAAYEAKQPAFMN

SEQ ID NO: 36 - protein, 201 aa, Artificial Sequence
  Synthesized - Modified LeuD (L31S H88V)
MAEKFIKHTGLVVPLDAANVDTDAIIPKQFSQKVTRTGFGAHLFNDWRFLDEKGQQPNPDFVLNFPQYQGASILLARENFGCGSSREVAPWALTDYGFKVVIAPSFADIFYGNSFNNQLLPVKLSDAEVDELFALVKANPGIHFDVDLEAQEVKAGEKTYRFTIDAFRRHCMMNGLDSIGLTLQHDDAIAAYEAKQPAFMN

SEQ ID NO: 37 - protein, 201 aa, Artificial Sequence
  Synthesized - Modified LeuD (L31S H88S)
MAEKFIKHTGLVVPLDAANVDTDAIIPKQFSQKVTRTGFGAHLFNDWRFLDEKGQQPNPDFVLNFPQYQGASILLARENFGCGSSRESAPWALTDYGFKVVIAPSFADIFYGNSFNNQLLPVKLSDAEVDELFALVKANPGIHFDVDLEAQEVKAGEKTYRFTIDAFRRHCMMNGLDSIGLTLQHDDAIAAYEAKQPAFMN

SEQ ID NO: 38 - protein, 10 aa, Artificial Sequence
  Synthesized - Variable Length C-Terminal Peptide
  MISC_FEATURE (1)..(2): Amino acids designated "Xaa" can be any naturally occurring amino acid.  Any one or all of amino acids designated "Xaa" at positions 1-2 can be present or absent.
  MISC_FEATURE (9)..(10): Amino acids designated "Xaa" can be any naturally occurring amino acid.  Any one or all of amino acids designated "Xaa" at positions 9-10 can be present or absent.
XXHHHHHHXX

SEQ ID NO: 39 - protein, 10 aa, Artificial Sequence
  Synthesized - Non-Variable C-Terminal Peptide
SSHHHHHHSS

SEQ ID NO: 40 - protein, 476 aa, Artificial Sequence
  Synthesized - LeuC' Subunit with C-Terminal Peptide
MAKTLYEKLFDAHVVYEAENETPLLYIDRHLVHEVTSPQAFDGLRAHGRPVRQPGKTFATMDHNVSTQTKDINACGEMARIQMQELIKNCKEFGVELYDLNHPYQGIVHVMGPEQGVTLPGMTIVCGDSHTATHGAFGALAFGIGTSEVEHVLATQTLKQGRAKTMKIEVQGKAAPGITAKDIVLAIIGKTGSAGGTGHVVEFCGEAIRDLSMEGRMTLCNMAIEMGAKAGLVAPDETTFNYVKGRLHAPKGKDFDDAVAYWKTLQTDEGATFDTVVTLQAEEISPQVTWGTNPGQVISVNDNIPDPASFADPVERASAEKALAYMGLKPGIPLTEVAIDKVFIGSCTNSRIEDLRAAAEIAKGRKVAPGVQALVVPGSGPVKAQAEAEGLDKIFIEAGFEWRLPGCSMCLAMNNDRLNPGERCASTSNRNFEGRQGRGGRTHLVSPAMAAAAAVTGHFADIRNIKSSHHHHHHSS